European Patent Specification EP 3 665 185 B1, published October 4, 2023. Title: VP-60 RECOMBINANT PROTEIN AND RELATIVE METHOD OF PRODUCTION AND PURIFICATION. Applicant: ISTITUTO ZOOPROFILATTICO SPERIMENTALE UMBRIA E MARCHE. The sequence listing filed with the application follows.

SEQUENCE LISTING (6 sequences)

SEQ ID NO: 1 - protein, 584 aa, Baculoviridae
  E-VP60-His6
MEGKPRADAPGTATTASVPGTTTDGMDPGVVASTDVVTADNVAASVATAGIGGPPQQVSPQESWRANFFYNDVFTWSVTDAPGSILYTVQHSPQNNPFTQVLSQMYAGWAGGMQFRFIVAGSGIFGGRLVCAIIPPGIQIQPGLEVRQFPHVVIDARSLEPVTITMPDLRPEMYHPTGNPGLVPTLVVSVYNNLINPFGGTTSAIQVTVETRPSEDFEFVLIRAPSSKTVDSVNPSWLLTTPVLTGAGSDNRWGAPIVGLQPVPGGFSTSNRHWNMNGETYGWSSPRFDDIDHPSGNVSYPTGSATNTIETWYANAGTATTNPISNVAPDGFPDMGAIPFSGSTIPTGAWVGFGQVWNASNGTPYVGTVQAYELGFASGAPSNVRPVTTTTGAQLVAKSIYGVAIAQNQSSAGIIFMSKGMVSTPGVAATTYTPQPSAIVTTPGTPVAAPIGKNTPIMFSAVVRRTGDVNAGPGSANGTQYGVGSQPLSVTLGLSLTNYSSALQPGQFFVWQLNFASGFMEIGLNTDGYFYAGTGAYSGMIELTDLIDVRPVGVRPNTSTLVFNLTGVATTGYSYVAGHHHHHH

SEQ ID NO: 2 - DNA, 1755 bp, Baculoviridae
  E-VP60-His/pOET2C
atggagggtaagcctcgggctgacgcccctggtaccgctaccacagcatctgttcctgggaccactaccgacggcatggacccaggggtggtggccagcactgacgttgtgacggctgacaacgttgcagcatctgttgccactgcggggattggaggaccaccacaacaggtctcacctcaagagtcttggcgtgcgaacttcttttacaatgatgtatttacctggtcagtcaccgatgcacccggtagcattctttacacagttcaacactccccgcaaaacaaccccttcacgcaggtgctgagccaaatgtatgctggttgggctggtggcatgcagtttagattcatagttgctgggtctggtatttttggcggaaggctcgtgtgtgcaatcataccacctgggatccagatacaacctgggcttgaggttagacagtttcctcatgttgtcatcgatgcacgctcacttgagccagtgactataacaatgcctgatcttcgtcctgaaatgtaccacccaacaggcaatcctggacttgtcccaacactcgtcgtgagtgtgtacaacaacttgatcaacccctttgggggtaccaccagtgcaattcaggttactgttgagactaggccaagtgaggactttgagtttgtgttgatccgcgcaccttcaagtaaaacagtggactcagtgaacccctcgtggctcttgacaactccggtcttgaccggtgctggttcagacaacagatggggtgcaccaattgtcgggctccagcccgtaccaggtggcttctccacttccaacaggcactggaacatgaatggtgaaacctacggttggtccagccccaggtttgacgacattgatcatccaagtggcaatgtatcctaccccactggtagtgcaaccaacaccattgagacctggtatgccaatgctggaacagctaccaccaacccaatctccaacgtagcaccagacgggtttcctgacatgggagccatcccgttcagtggctcaaccatcccgactggtgcctgggttgggtttgggcaggtgtggaacgcctccaatggcaccccatacgtggggaccgttcaggcgtacgagctggggttcgcaagcggggccccgtccaacgttcgtcctgtcacaacaaccacgggtgcgcagctggttgcaaagtcgatctatggggttgccattgcccaaaaccaatccagtgctggcattatcttcatgtcgaaagggatggtctcaacacctggggtggctgccacaacatacaccccgcaaccaagcgcaattgtcacaacacctggaacacctgtggctgcacccattggcaagaatacacctattatgttcagtgcagtcgtgcggaggactggtgatgtgaacgccggtcctgggtccgctaacggcacacagtatggcgttggctcgcagccattgtcagtaacacttggactgtccctgacaaactactcctccgcacttcaacctggccagttctttgtgtggcaactcaacttcgcttctggcttcatggagattggtttgaatacagatggttacttttatgcagggactggtgcttactcaggcatgattgaattgacagacctcattgatgtgcggcccgtgggagtccggccaaacacgagcacactcgtgttcaaccttaccggagtggccaccactggatattcctatgtcgccggtcatcatcaccatcaccattga

SEQ ID NO: 3 - DNA, 40 bp, Baculoviridae
  EBHS-VP60-F
gatagtctcgaggccaccatggagggtaagcctcgggctg

SEQ ID NO: 4 - DNA, 32 bp, Baculoviridae
  EBHS-VP60/NgoMiv-R
cctaggccggcgacataggaatatccagtggt

SEQ ID NO: 5 - DNA, 21 bp, Baculoviridae
  EBHS-VP60/ApaLI-R
gagcccgacaattggtgcacc

SEQ ID NO: 6 - DNA, 21 bp, Baculoviridae
  EBHS-VP60/ApaLI-F
cagacaacaggtggggtgcac